European Patent Application EP 4 778 943 A1, published July 22, 2026. Title: 长效甲状旁腺激素受体激动剂融合蛋白及其应用. Applicant: 上海才致药成生物科技有限公司. The sequence listing filed with the application follows.

SEQUENCE LISTING (40 sequences)

SEQ ID NO: 1 - protein, 122 aa, synthetic construct
EVQLLESGGGLVQPGGSLRLSCAASGFTFSSYAMSWVRQAPGKGLEWVSGITGSGGSTYYADSVKGRFTISRDNSKNTLYLQMNSLRAEDTAVYYCAKDPGTTVIMSWFDPWGQGTLVTVSS

SEQ ID NO: 2 - protein, 108 aa, synthetic construct
EIVLTQSPGTLSLSPGERATLSCRASQSVRGRYLAWYQQKPGQAPRLLIYGASSRATGIPDRFSGSGSGTDFTLTISRLEPEDFAVFYCQQYGSSPRTFGQGTKVEIK

SEQ ID NO: 3 - protein, 121 aa, synthetic construct
QVQLVQSGAEVKKPGSSVKVSCKASGYAFTNYYIEWVRQAPGQGLEWMGVINPGWGDTNYNEKFKGRVTITADKSTSTAYMELSSLRSEDTAVYYCARRDTAHGYYALDPWGQGTTVTVSS

SEQ ID NO: 4 - protein, 107 aa, synthetic construct
DIQMTQSPSSLSASVGDRVTITCKASQNVGTNVAWYQQKPGKAPKLLIYSASYRYSGVPSRFSGSGSGTDFTLTISSLQPEDFATYYCQQYWDYPLTFGGGTKVEIK

SEQ ID NO: 5 - protein, 34 aa, synthetic construct
SVSEIQLMHNLGKHLNSMERVEWLRKKLQDVHNF

SEQ ID NO: 6 - protein, 229 aa, synthetic construct
ESKYGPPCPPCPAPEFLGGPSVFLFPPKPKDTLMISRTPEVTCVVVDVSQEDPEVQFNWYVDGVEVHNAKTKPREEQFNSTYRVVSVLTVLHQDWLNGKEYKCKVSNKGLPSSIEKTISKAKGQPREPQVYTLPPSQEEMTKNQVSLTCLVKGFYPSDIAVEWESNGQPENNYKTTPPVLDSDGSFFLYSRLTVDKSRWQEGNVFSCSVMHEALHNHYTQKSLSLSLGK

SEQ ID NO: 7 - protein, 229 aa, synthetic construct
ESKYGPPCPPCPAPEFLGGPSVFLFPPKPKDTLMISRTPEVTCVVVDVSQEDPEVQFNWYVDGVEVHNAKTKPREEQFNSTYRVVSVLTVLHQDWLNGKEYKCKVSNKGLPSSIEKTISKAKGQPREPQVYTLPPSQEEMTKNQVSLSCAVKGFYPSDIAVEWESNGQPENNYKTTPPVLDSDGSFFLVSRLTVDKSRWQEGNVFSCSVMHEALHNHYTQKSLSLSLGK

SEQ ID NO: 8 - protein, 229 aa, synthetic construct
ESKYGPPCPPCPAPEFLGGPSVFLFPPKPKDTLMISRTPEVTCVVVDVSQEDPEVQFNWYVDGVEVHNAKTKPREEQFNSTYRVVSVLTVLHQDWLNGKEYKCKVSNKGLPSSIEKTISKAKGQPREPQVYTLPPSQEEMTKNQVSLWCLVKGFYPSDIAVEWESNGQPENNYKTTPPVLDSDGSFFLYSRLTVDKSRWQEGNVFSCSVMHEALHNHYTQKSLSLSLGK

SEQ ID NO: 9 - protein, 5 aa, synthetic construct
GGGGS

SEQ ID NO: 10 - protein, 10 aa, synthetic construct
GGGGSGGGGS

SEQ ID NO: 11 - protein, 15 aa, synthetic construct
GGGGSGGGGSGGGGS

SEQ ID NO: 12 - protein, 20 aa, synthetic construct
GGGGSGGGGSGGGGSGGGGS

SEQ ID NO: 13 - protein, 17 aa, synthetic construct
MRAWIFFLLCLAGRALA

SEQ ID NO: 14 - protein, 98 aa, synthetic construct
ASTKGPSVFPLAPCSRSTSESTAALGCLVKDYFPEPVTVSWNSGALTSGVHTFPAVLQSSGLYSLSSVVTVPSSSLGTKTYTCNVDHKPSNTKVDKRV

SEQ ID NO: 15 - protein, 107 aa, synthetic construct [sequence omitted]

SEQ ID NO: 16 - protein, 5 aa, synthetic construct
SYAMS

SEQ ID NO: 17 - protein, 17 aa, synthetic construct
GITGSGGSTYYADSVKG

SEQ ID NO: 18 - protein, 13 aa, synthetic construct
DPGTTVIMSWFDP

SEQ ID NO: 19 - protein, 12 aa, synthetic construct
RASQSVRGRYLA

SEQ ID NO: 20 - protein, 7 aa, synthetic construct
GASSRAT

SEQ ID NO: 21 - protein, 9 aa, synthetic construct
QQYGSSPRT

SEQ ID NO: 22 - protein, 5 aa, synthetic construct
NYYIE

SEQ ID NO: 23 - protein, 17 aa, synthetic construct
VINPGWGDTNYNEKFKG

SEQ ID NO: 24 - protein, 12 aa, synthetic construct
RDTAHGYYALDP

SEQ ID NO: 25 - protein, 11 aa, synthetic construct
KASQNVGTNVA

SEQ ID NO: 26 - protein, 7 aa, synthetic construct
SASYRYS

SEQ ID NO: 27 - protein, 9 aa, synthetic construct
QQYWDYPLT

SEQ ID NO: 28 - protein, 4 aa, synthetic construct
GGGS

SEQ ID NO: 29 - protein, 5 aa, synthetic construct
EAAAK

SEQ ID NO: 30 - protein, 34 aa, synthetic construct
  MOD_RES 29: note = Aib
AVSEHQLLHDKGKSIQDLRRRELLEKLLXKLHTA

SEQ ID NO: 31 - protein, 11 aa, synthetic construct
SVAEIALMHQR

SEQ ID NO: 32 - protein, 20 aa, synthetic construct
SVSEIQLMHNLGKHLNSMER

SEQ ID NO: 33 - protein, 37 aa, synthetic construct
SVSEIQLMHNLGKHLNSMERVEWLRKKLQDVHNFVAL

SEQ ID NO: 34 - protein, 38 aa, synthetic construct
SVSEIQLMHNLGKHLNSMERVEWLRKKLQDVHNFVALG

SEQ ID NO: 35 - protein, 41 aa, synthetic construct
SVSEIQLMHNLGKHLNSMERVEWLRKKLQDVHNFVALGAPL

SEQ ID NO: 36 - protein, 36 aa, synthetic construct
AVSEHQLLHDKGKSIQDLRRRFFLHHLIAEIHTAEI

SEQ ID NO: 37 - protein, 84 aa, synthetic construct
SVSEIQLMHNLGKHLNSMERVEWLRKKLQDVHNFVALGAPLAPRDAGSQRPRKKEDNVLVESHEKSLGEADKADVNVLTKAKSQ

SEQ ID NO: 38 - protein, 14 aa, synthetic construct
AVAEIQLMHQRAKW

SEQ ID NO: 39 - protein, 232 aa, synthetic construct
EPKSCDKTHTCPPCPAPEAAGGPSVFLFPPKPKDTLMISRTPEVTCVVVDVSHEDPEVKFNWYVDGVEVHNAKTKPREEQYNSTYRVVSVLTVLHQDWLNGKEYKCKVSNKALPAPIEKTISKAKGQPREPQVYTLPPSREEMTKNQVSLSCAVKGFYPSDIAVEWESNGQPENNYKTTPPVLDSDGSFFLVSKLTVDKSRWQQGNVFSCSVMHEALHNHYTQKSLSLSPGK

SEQ ID NO: 40 - protein, 232 aa, synthetic construct
EPKSCDKTHTCPPCPAPEAAGGPSVFLFPPKPKDTLMISRTPEVTCVVVDVSHEDPEVKFNWYVDGVEVHNAKTKPREEQYNSTYRVVSVLTVLHQDWLNGKEYKCKVSNKALPAPIEKTISKAKGQPREPQVYTLPPSREEMTKNQVSLWCLVKGFYPSDIAVEWESNGQPENNYKTTPPVLDSDGSFFLYSKLTVDKSRWQQGNVFSCSVMHEALHNHYTQKSLSLSPGK